European Patent Application EP 4 212 625 A1, published July 19, 2023. Title: Polypeptide having 4-aminobenzoic acid hydroxylation activity and use thereof. Applicant: KAO CORPORATION. The sequence listing filed with the application follows.

SEQUENCE LISTING (50 sequences)

SEQ ID NO: 1 - DNA, 1176 bp, Caulobacter vibrioides
  CDS (1)..(1173): Codon-optimized oligonucleotide
atgcgcactcaggtggctatcgtaggagcaggcccagctggcctgttcttgggccatctcctccgtcaagctggtgtggacgtcgtgattctggaacgcaaagaccgtgcttatgtcgaaggccgagttcgggctggtgtcctggaacgtatcacggtggagctgatggagcgtcttggtgtggatgagcgaatgcgccgagagggcttggtgcatgctggcgctaatcttgcgtctgatggcgagatgttccgtatcgacatggcagagctcacgggtggttccaccgtcatggtttacggccaacaggaggtgatgaaggacctgtttgatgcagcagagcagcgcgatctgcgaattgtctttgacgccgatgcagtgcgtctgcacgatgtggaaggcgaacgtcctcacatcacctggcgcaaagacggggcagaacaccgcctggactgcgatttcattgccggctgcgacggctaccacggagtttctcgtgcgaccattcccgataaggttctcaagaccttcgaacgggtgtatccctttgggtggttgggaatcctggctgaagcacctccgtgtgaccacgagttgatctactcgaaccatgatcgcggttttgccctggcgtcgatgcgctcaccgacacgctcccgctattacgtgcagtgctcactcgacgatcgcctcgaggattggtccgatgaacggttctgggatgaagtttcggttcgcctgggaccggaagcagccgctcggatcgttcgcgcaccttccttcgagaagagcattgccccacttcgctccttcgtttccgagcctatgcggtatggccgccttttcctcgcgggtgatgcggctcatatcgttccacccactggagcgaaagggatgaacttggccgtatcagacgtcatcatgctgtccgaagccctggtcgaacactaccacgaacgctcttccgctggtatcgatggttacagcgcacgtgcacttgcccgcgtctggaaggcggagcgtttcagctggtggtttacctcccttactcaccgcttcccagaccaggacggcttcgaccgcaagatgcaagtcgccgaattggcatacatcaagggttctcgcgctgcccaggtcaccctggcggagaactacgtaggactgccactcgtataa

SEQ ID NO: 2 - protein, 391 aa, Caulobacter vibrioides
MRTQVAIVGAGPAGLFLGHLLRQAGVDVVILERKDRAYVEGRVRAGVLERITVELMERLGVDERMRREGLVHAGANLASDGEMFRIDMAELTGGSTVMVYGQQEVMKDLFDAAEQRDLRIVFDADAVRLHDVEGERPHITWRKDGAEHRLDCDFIAGCDGYHGVSRATIPDKVLKTFERVYPFGWLGILAEAPPCDHELIYSNHDRGFALASMRSPTRSRYYVQCSLDDRLEDWSDERFWDEVSVRLGPEAAARIVRAPSFEKSIAPLRSFVSEPMRYGRLFLAGDAAHIVPPTGAKGMNLAVSDVIMLSEALVEHYHERSSAGIDGYSARALARVWKAERFSWWFTSLTHRFPDQDGFDRKMQVAELAYIKGSRAAQVTLAENYVGLPLV

SEQ ID NO: 3 - DNA, 42 bp, Artificial Sequence
  Synthetic oligonucleotide
tattaattaaatgcgcgttttaattattgataattatgattc

SEQ ID NO: 4 - DNA, 45 bp, Artificial Sequence
  Synthetic oligonucleotide
ttgcggccgcttgtttaaacctccttacagaaaaatggttgggcg

SEQ ID NO: 5 - DNA, 33 bp, Artificial Sequence
  Synthetic oligonucleotide
aaatttaaacctcctttacagaaaaatggttgg

SEQ ID NO: 6 - DNA, 28 bp, Artificial Sequence
  Synthetic oligonucleotide
ggaggtttaaacaagcggccgcgatatc

SEQ ID NO: 7 - DNA, 35 bp, Artificial Sequence
  Synthetic oligonucleotide
aggaggtttaaatttatgcgcactcaggtggctat

SEQ ID NO: 8 - DNA, 35 bp, Artificial Sequence
  Synthetic oligonucleotide
cttgtttaaacctccttatacgagtggcagtccta

SEQ ID NO: 9 - DNA, 31 bp, Artificial Sequence
  Synthetic oligonucleotide
gctatcaaaacattcggcacattggttttcc

SEQ ID NO: 10 - DNA, 29 bp, Artificial Sequence
  Synthetic oligonucleotide
ggaagatgcgtgatctgatccttcaactc

SEQ ID NO: 11 - DNA, 24 bp, Artificial Sequence
  Synthetic oligonucleotide
ttacagaaaaatggttgggcgcaa

SEQ ID NO: 12 - DNA, 22 bp, Artificial Sequence
  Synthetic oligonucleotide
atgcgcactcaggtggctatcg

SEQ ID NO: 13 - DNA, 342 bp, Artificial Sequence
  Synthetic oligonucleotide
tacgtacctgcaggtagcgtgtcagtaggcgcgtagggtaagtggggtagcggcttgttagatatcttgaaatcggctttcaacagcattgatttcgatgtatttagctggccgttaccctgcgaatgtccacagggtagctggtagtttgaaaatcaacgccgttgcccttaggattcagtaactggcacattttgtaatgcgctagatctgtgtgctcagtcttccaggctgcttatcacagtgaaagcaaaaccaattcgtggctgcgaaagtcgtagccaccacgaagtccaaaggaggatctaaattatgaataatataaaaggaggaattaattaa

SEQ ID NO: 14 - DNA, 36 bp, Artificial Sequence
  Synthetic oligonucleotide
accatttttctgtaatacgtacctgcaggtagcgtg

SEQ ID NO: 15 - DNA, 35 bp, Artificial Sequence
  Synthetic oligonucleotide
cacctgagtgcgcatttaattaattcctcctttta

SEQ ID NO: 16 - DNA, 29 bp, Artificial Sequence
  Synthetic oligonucleotide
gcttgttagatatcttgaaatcggctttc

SEQ ID NO: 17 - DNA, 27 bp, Artificial Sequence
  Synthetic oligonucleotide
gcttattgtgaaggccgagttcgggct

SEQ ID NO: 18 - DNA, 27 bp, Artificial Sequence
  Synthetic oligonucleotide
gccttcacaataagcacggtctttgcg

SEQ ID NO: 19 - DNA, 27 bp, Artificial Sequence
  Synthetic oligonucleotide
ggccgactccgggctggtgtcctggaa

SEQ ID NO: 20 - DNA, 27 bp, Artificial Sequence
  Synthetic oligonucleotide
agcccggagtcggccttcgacataagc

SEQ ID NO: 21 - DNA, 27 bp, Artificial Sequence
  Synthetic oligonucleotide
ggccgacatcgggctggtgtcctggaa

SEQ ID NO: 22 - DNA, 27 bp, Artificial Sequence
  Synthetic oligonucleotide
agcccgatgtcggccttcgacataagc

SEQ ID NO: 23 - DNA, 27 bp, Artificial Sequence
  Synthetic oligonucleotide
ggcgaggttttccgtatcgacatggca

SEQ ID NO: 24 - DNA, 27 bp, Artificial Sequence
  Synthetic oligonucleotide
acggaaaacctcgccatcagacgcaag

SEQ ID NO: 25 - DNA, 27 bp, Artificial Sequence
  Synthetic oligonucleotide
ggcgagggtttccgtatcgacatggca

SEQ ID NO: 26 - DNA, 27 bp, Artificial Sequence
  Synthetic oligonucleotide
acggaaaccctcgccatcagacgcaag

SEQ ID NO: 27 - DNA, 27 bp, Artificial Sequence
  Synthetic oligonucleotide
ggcgagttcttccgtatcgacatggca

SEQ ID NO: 28 - DNA, 27 bp, Artificial Sequence
  Synthetic oligonucleotide
acggaagaactcgccatcagacgcaag

SEQ ID NO: 29 - DNA, 27 bp, Artificial Sequence
  Synthetic oligonucleotide
gaggtggcaaaggacctgtttgatgca

SEQ ID NO: 30 - DNA, 27 bp, Artificial Sequence
  Synthetic oligonucleotide
gtcctttgccacctcctgttggccgta

SEQ ID NO: 31 - DNA, 27 bp, Artificial Sequence
  Synthetic oligonucleotide
gaggtgtgtaaggacctgtttgatgca

SEQ ID NO: 32 - DNA, 27 bp, Artificial Sequence
  Synthetic oligonucleotide
gtccttacacacctcctgttggccgta

SEQ ID NO: 33 - DNA, 27 bp, Artificial Sequence
  Synthetic oligonucleotide
gaggtgattaaggacctgtttgatgca

SEQ ID NO: 34 - DNA, 27 bp, Artificial Sequence
  Synthetic oligonucleotide
gtccttaatcacctcctgttggccgta

SEQ ID NO: 35 - DNA, 27 bp, Artificial Sequence
  Synthetic oligonucleotide
gaggtgacaaaggacctgtttgatgca

SEQ ID NO: 36 - DNA, 27 bp, Artificial Sequence
  Synthetic oligonucleotide
gtcctttgtcacctcctgttggccgta

SEQ ID NO: 37 - DNA, 27 bp, Artificial Sequence
  Synthetic oligonucleotide
gaacgggcatatccctttgggtggttg

SEQ ID NO: 38 - DNA, 27 bp, Artificial Sequence
  Synthetic oligonucleotide
gggatatgcccgttcgaaggtcttgag

SEQ ID NO: 39 - DNA, 27 bp, Artificial Sequence
  Synthetic oligonucleotide
agcattgttccacttcgctccttcgtt

SEQ ID NO: 40 - DNA, 27 bp, Artificial Sequence
  Synthetic oligonucleotide
aagtggaacaatgctcttctcgaagga

SEQ ID NO: 41 - DNA, 27 bp, Artificial Sequence
  Synthetic oligonucleotide
agcattttcccacttcgctccttcgtt

SEQ ID NO: 42 - DNA, 27 bp, Artificial Sequence
  Synthetic oligonucleotide
aagtgggaaaatgctcttctcgaagga

SEQ ID NO: 43 - DNA, 27 bp, Artificial Sequence
  Synthetic oligonucleotide
tggtggctcacctcccttactcaccgc

SEQ ID NO: 44 - DNA, 27 bp, Artificial Sequence
  Synthetic oligonucleotide
ggaggtgagccaccagctgaaacgctc

SEQ ID NO: 45 - DNA, 27 bp, Artificial Sequence
  Synthetic oligonucleotide
cgcaaggttcaagtcgccgaattggca

SEQ ID NO: 46 - DNA, 27 bp, Artificial Sequence
  Synthetic oligonucleotide
gacttgaaccttgcggtcgaagccgtc

SEQ ID NO: 47 - DNA, 27 bp, Artificial Sequence
  Synthetic oligonucleotide
cgcaagctccaagtcgccgaattggca

SEQ ID NO: 48 - DNA, 27 bp, Artificial Sequence
  Synthetic oligonucleotide
gacttggagcttgcggtcgaagccgtc

SEQ ID NO: 49 - DNA, 27 bp, Artificial Sequence
  Synthetic oligonucleotide
gcatacttcaagggttctcgcgctgcc

SEQ ID NO: 50 - DNA, 27 bp, Artificial Sequence
  Synthetic oligonucleotide
acccttgaagtatgccaattcggcgac